European Patent Application EP 4 180 533 A1, published May 17, 2023. Title: Highly-Multiplexed Fluorescent Imaging. Applicant: The Board of Trustees of the Leland Stanford Junior University. Application US. The sequence listing filed with the application follows.

SEQUENCE LISTING (94 sequences)

SEQ ID NO: 1 - DNA, 15 bp, synthetic construct
  misc_feature 1..15: note = synthetic nucleic acid
  source 1..15: mol_type = other DNA
ttagacaactttagt

SEQ ID NO: 2 - DNA, 15 bp, synthetic construct
  misc_feature 1..15: note = synthetic nucleic acid
  source 1..15: mol_type = other DNA
catcaggatttggta

SEQ ID NO: 3 - DNA, 15 bp, synthetic construct
  misc_feature 1..15: note = synthetic nucleic acid
  source 1..15: mol_type = other DNA
cgctcctcatgataa

SEQ ID NO: 4 - DNA, 13 bp, synthetic construct
  misc_feature 1..13: note = synthetic nucleic acid
  source 1..13: mol_type = other DNA
cggccatccatta

SEQ ID NO: 5 - DNA, 15 bp, synthetic construct
  misc_feature 1..15: note = synthetic nucleic acid
  source 1..15: mol_type = other DNA
ggctgattaccctct

SEQ ID NO: 6 - DNA, 15 bp, synthetic construct
  misc_feature 1..15: note = synthetic nucleic acid
  source 1..15: mol_type = other DNA
tagcattgtgtaggt

SEQ ID NO: 7 - DNA, 17 bp, synthetic construct
  misc_feature 1..17: note = synthetic nucleic acid
  source 1..17: mol_type = other DNA
gaatcttatagaatcgc

SEQ ID NO: 8 - DNA, 15 bp, synthetic construct
  misc_feature 1..15: note = synthetic nucleic acid
  source 1..15: mol_type = other DNA
cttataagtagacgc

SEQ ID NO: 9 - DNA, 14 bp, synthetic construct
  misc_feature 1..14: note = synthetic nucleic acid
  source 1..14: mol_type = other DNA
ctgggcgagatatg

SEQ ID NO: 10 - DNA, 11 bp, synthetic construct
  misc_feature 1..11: note = synthetic nucleic acid
  source 1..11: mol_type = other DNA
ctcggcccgat

SEQ ID NO: 11 - DNA, 17 bp, synthetic construct
  misc_feature 1..17: note = synthetic nucleic acid
  source 1..17: mol_type = other DNA
agattactactcataca

SEQ ID NO: 12 - DNA, 15 bp, synthetic construct
  misc_feature 1..15: note = synthetic nucleic acid
  source 1..15: mol_type = other DNA
gctctctgacttaga

SEQ ID NO: 13 - DNA, 15 bp, synthetic construct
  misc_feature 1..15: note = synthetic nucleic acid
  source 1..15: mol_type = other DNA
atcacggataatgtc

SEQ ID NO: 14 - DNA, 17 bp, synthetic construct
  misc_feature 1..17: note = synthetic nucleic acid
  source 1..17: mol_type = other DNA
agtactaatagtagtga

SEQ ID NO: 15 - DNA, 12 bp, synthetic construct
  misc_feature 1..12: note = synthetic nucleic acid
  source 1..12: mol_type = other DNA
tggcattctggc

SEQ ID NO: 16 - DNA, 14 bp, synthetic construct
  misc_feature 1..14: note = synthetic nucleic acid
  source 1..14: mol_type = other DNA
ctcaggttcgagtc

SEQ ID NO: 17 - DNA, 15 bp, synthetic construct
  misc_feature 1..15: note = synthetic nucleic acid
  source 1..15: mol_type = other DNA
ctctggtaggatgta

SEQ ID NO: 18 - DNA, 13 bp, synthetic construct
  misc_feature 1..13: note = synthetic nucleic acid
  source 1..13: mol_type = other DNA
cactttgccgtgc

SEQ ID NO: 19 - DNA, 15 bp, synthetic construct
  misc_feature 1..15: note = synthetic nucleic acid
  source 1..15: mol_type = other DNA
gatacgaggcgttat

SEQ ID NO: 20 - DNA, 15 bp, synthetic construct
  misc_feature 1..15: note = synthetic nucleic acid
  source 1..15: mol_type = other DNA
cacagactcctttgg

SEQ ID NO: 21 - DNA, 13 bp, synthetic construct
  misc_feature 1..13: note = synthetic nucleic acid
  source 1..13: mol_type = other DNA
attttcccgcacg

SEQ ID NO: 22 - DNA, 15 bp, synthetic construct
  misc_feature 1..15: note = synthetic nucleic acid
  source 1..15: mol_type = other DNA
atgcaatcacctggt

SEQ ID NO: 23 - DNA, 15 bp, synthetic construct
  misc_feature 1..15: note = synthetic nucleic acid
  source 1..15: mol_type = other DNA
gaagtttacgggata

SEQ ID NO: 24 - DNA, 15 bp, synthetic construct
  misc_feature 1..15: note = synthetic nucleic acid
  source 1..15: mol_type = other DNA
actaagcgagtacac

SEQ ID NO: 25 - DNA, 15 bp, synthetic construct
  misc_feature 1..15: note = synthetic nucleic acid
  source 1..15: mol_type = other DNA
aatctgttgaaatca

SEQ ID NO: 26 - DNA, 15 bp, synthetic construct
  misc_feature 1..15: note = synthetic nucleic acid
  source 1..15: mol_type = other DNA
gtagtcctaaaccat

SEQ ID NO: 27 - DNA, 12 bp, synthetic construct
  misc_feature 1..12: note = synthetic nucleic acid
  source 1..12: mol_type = other DNA
cggcgaggagta

SEQ ID NO: 28 - DNA, 12 bp, synthetic construct
  misc_feature 1..12: note = synthetic nucleic acid
  source 1..12: mol_type = other DNA
acgccggtaggt

SEQ ID NO: 29 - DNA, 15 bp, synthetic construct
  misc_feature 1..15: note = synthetic nucleic acid
  source 1..15: mol_type = other DNA
ccgactaatgggaga

SEQ ID NO: 30 - DNA, 15 bp, synthetic construct
  misc_feature 1..15: note = synthetic nucleic acid
  source 1..15: mol_type = other DNA
atcgtaacacatcca

SEQ ID NO: 31 - DNA, 17 bp, synthetic construct
  misc_feature 1..17: note = synthetic nucleic acid
  source 1..17: mol_type = other DNA
cttagaatatcttagcg

SEQ ID NO: 32 - DNA, 15 bp, synthetic construct
  misc_feature 1..15: note = synthetic nucleic acid
  source 1..15: mol_type = other DNA
gaatattcatctgcg

SEQ ID NO: 33 - DNA, 14 bp, synthetic construct
  misc_feature 1..14: note = synthetic nucleic acid
  source 1..14: mol_type = other DNA
ctatcgtccgtgca

SEQ ID NO: 34 - DNA, 12 bp, synthetic construct
  misc_feature 1..12: note = synthetic nucleic acid
  source 1..12: mol_type = other DNA
gagccgggctag

SEQ ID NO: 35 - DNA, 15 bp, synthetic construct
  misc_feature 1..15: note = synthetic nucleic acid
  source 1..15: mol_type = other DNA
cgagagactgaatct

SEQ ID NO: 36 - DNA, 15 bp, synthetic construct
  misc_feature 1..15: note = synthetic nucleic acid
  source 1..15: mol_type = other DNA
tagtgcctattacag

SEQ ID NO: 37 - DNA, 15 bp, synthetic construct
  misc_feature 1..15: note = synthetic nucleic acid
  source 1..15: mol_type = other DNA
tcatgattatcatca

SEQ ID NO: 38 - DNA, 15 bp, synthetic construct
  misc_feature 1..15: note = synthetic nucleic acid
  source 1..15: mol_type = other DNA
accgtaagaccgctt

SEQ ID NO: 39 - DNA, 15 bp, synthetic construct
  misc_feature 1..15: note = synthetic nucleic acid
  source 1..15: mol_type = other DNA
gagtccaagctcagc

SEQ ID NO: 40 - DNA, 15 bp, synthetic construct
  misc_feature 1..15: note = synthetic nucleic acid
  source 1..15: mol_type = other DNA
gagaccatcctacat

SEQ ID NO: 41 - DNA, 13 bp, synthetic construct
  misc_feature 1..13: note = synthetic nucleic acid
  source 1..13: mol_type = other DNA
gtgaaacggcacg

SEQ ID NO: 42 - DNA, 15 bp, synthetic construct
  misc_feature 1..15: note = synthetic nucleic acid
  source 1..15: mol_type = other DNA
ctatgctccgcaata

SEQ ID NO: 43 - DNA, 15 bp, synthetic construct
  misc_feature 1..15: note = synthetic nucleic acid
  source 1..15: mol_type = other DNA
gtgtctgaggaaacc

SEQ ID NO: 44 - DNA, 13 bp, synthetic construct
  misc_feature 1..13: note = synthetic nucleic acid
  source 1..13: mol_type = other DNA
taaaagggcgtgc

SEQ ID NO: 45 - DNA, 15 bp, synthetic construct
  misc_feature 1..15: note = synthetic nucleic acid
  source 1..15: mol_type = other DNA
tacgttagtggacca

SEQ ID NO: 46 - DNA, 15 bp, synthetic construct
  misc_feature 1..15: note = synthetic nucleic acid
  source 1..15: mol_type = other DNA
cttcaaatgccctat

SEQ ID NO: 47 - DNA, 15 bp, synthetic construct
  misc_feature 1..15: note = synthetic nucleic acid
  source 1..15: mol_type = other DNA
tgattcgctcatgtg

SEQ ID NO: 48 - DNA, 33 bp, synthetic construct
  misc_feature 1..33: note = synthetic nucleic acid
  source 1..33: mol_type = other DNA
atagcagtccagcgccccactaaagttgtctaa

SEQ ID NO: 49 - DNA, 33 bp, synthetic construct
  misc_feature 1..33: note = synthetic nucleic acid
  source 1..33: mol_type = other DNA
atagcagtccagaacgactaccaaatcctgatg

SEQ ID NO: 50 - DNA, 33 bp, synthetic construct
  misc_feature 1..33: note = synthetic nucleic acid
  source 1..33: mol_type = other DNA
atagcagtccagctattatcatgaggagcggcg

SEQ ID NO: 51 - DNA, 33 bp, synthetic construct
  misc_feature 1..33: note = synthetic nucleic acid
  source 1..33: mol_type = other DNA
atagcagtccaggatcttaatggatggccgcag

SEQ ID NO: 52 - DNA, 33 bp, synthetic construct
  misc_feature 1..33: note = synthetic nucleic acid
  source 1..33: mol_type = other DNA
atagcagtccagcgggtgagagggtaatcagcc

SEQ ID NO: 53 - DNA, 33 bp, synthetic construct
  misc_feature 1..33: note = synthetic nucleic acid
  source 1..33: mol_type = other DNA
atagcagtccaggtgtccacctacacaatgcta

SEQ ID NO: 54 - DNA, 33 bp, synthetic construct
  misc_feature 1..33: note = synthetic nucleic acid
  source 1..33: mol_type = other DNA
atagcagtccagtcgggcgattctataagattc

SEQ ID NO: 55 - DNA, 33 bp, synthetic construct
  misc_feature 1..33: note = synthetic nucleic acid
  source 1..33: mol_type = other DNA
atagcagtccagcgcattgcgtctacttataag

SEQ ID NO: 56 - DNA, 33 bp, synthetic construct
  misc_feature 1..33: note = synthetic nucleic acid
  source 1..33: mol_type = other DNA
atagcagtccagttaaacgcatatctcgcccag

SEQ ID NO: 57 - DNA, 33 bp, synthetic construct
  misc_feature 1..33: note = synthetic nucleic acid
  source 1..33: mol_type = other DNA
atagcagtccagtcattcgtagatcgggccgag

SEQ ID NO: 58 - DNA, 33 bp, synthetic construct
  misc_feature 1..33: note = synthetic nucleic acid
  source 1..33: mol_type = other DNA
atagcagtccagttactgtatgagtagtaatct

SEQ ID NO: 59 - DNA, 33 bp, synthetic construct
  misc_feature 1..33: note = synthetic nucleic acid
  source 1..33: mol_type = other DNA
atagcagtccaggctacctctaagtcagagagc

SEQ ID NO: 60 - DNA, 33 bp, synthetic construct
  misc_feature 1..33: note = synthetic nucleic acid
  source 1..33: mol_type = other DNA
atagcagtccaggctcgtgacattatccgtgat

SEQ ID NO: 61 - DNA, 33 bp, synthetic construct
  misc_feature 1..33: note = synthetic nucleic acid
  source 1..33: mol_type = other DNA
atagcagtccagtttctcactactattagtact

SEQ ID NO: 62 - DNA, 33 bp, synthetic construct
  misc_feature 1..33: note = synthetic nucleic acid
  source 1..33: mol_type = other DNA
atagcagtccagccttgtttcgccagaatgcca

SEQ ID NO: 63 - DNA, 33 bp, synthetic construct
  misc_feature 1..33: note = synthetic nucleic acid
  source 1..33: mol_type = other DNA
atagcagtccagctcttccgactcgaacctgag

SEQ ID NO: 64 - DNA, 33 bp, synthetic construct
  misc_feature 1..33: note = synthetic nucleic acid
  source 1..33: mol_type = other DNA
atagcagtccagttagcctacatcctaccagag

SEQ ID NO: 65 - DNA, 33 bp, synthetic construct
  misc_feature 1..33: note = synthetic nucleic acid
  source 1..33: mol_type = other DNA
atagcagtccagcatggcctgcacggcaaagtg

SEQ ID NO: 66 - DNA, 33 bp, synthetic construct
  misc_feature 1..33: note = synthetic nucleic acid
  source 1..33: mol_type = other DNA
atagcagtccagatggcaataacgcctcgtatc

SEQ ID NO: 67 - DNA, 33 bp, synthetic construct
  misc_feature 1..33: note = synthetic nucleic acid
  source 1..33: mol_type = other DNA
atagcagtccaggaagcgccaaaggagtctgtg

SEQ ID NO: 68 - DNA, 33 bp, synthetic construct
  misc_feature 1..33: note = synthetic nucleic acid
  source 1..33: mol_type = other DNA
atagcagtccagtccgtctccgtgcgggaaaat

SEQ ID NO: 69 - DNA, 33 bp, synthetic construct
  misc_feature 1..33: note = synthetic nucleic acid
  source 1..33: mol_type = other DNA
atagcagtccagatactaaccaggtgattgcat

SEQ ID NO: 70 - DNA, 33 bp, synthetic construct
  misc_feature 1..33: note = synthetic nucleic acid
  source 1..33: mol_type = other DNA
atagcagtccaggcgcactatcccgtaaacttc

SEQ ID NO: 71 - DNA, 34 bp, synthetic construct
  misc_feature 1..34: note = synthetic nucleic acid
  source 1..34: mol_type = other DNA
atagcagtccaggggcatgtgtactcgcttagtr

SEQ ID NO: 72 - DNA, 35 bp, synthetic construct
  misc_feature 1..35: note = synthetic nucleic acid
  source 1..35: mol_type = other DNA
atagcagtccaggcggggtgatttcaacagattaa

SEQ ID NO: 73 - DNA, 35 bp, synthetic construct
  misc_feature 1..35: note = synthetic nucleic acid
  source 1..35: mol_type = other DNA
atagcagtccagttgctgatggtttaggactacgg

SEQ ID NO: 74 - DNA, 35 bp, synthetic construct
  misc_feature 1..35: note = synthetic nucleic acid
  source 1..35: mol_type = other DNA
atagcagtccaggataatagtactcctcgccgcaa

SEQ ID NO: 75 - DNA, 35 bp, synthetic construct
  misc_feature 1..35: note = synthetic nucleic acid
  source 1..35: mol_type = other DNA
atagcagtccagctagaattacctaccggcgtcgg

SEQ ID NO: 76 - DNA, 35 bp, synthetic construct
  misc_feature 1..35: note = synthetic nucleic acid
  source 1..35: mol_type = other DNA
atagcagtccaggcccactctcccattagtcggaa

SEQ ID NO: 77 - DNA, 35 bp, synthetic construct
  misc_feature 1..35: note = synthetic nucleic acid
  source 1..35: mol_type = other DNA
atagcagtccagcacaggtggatgtgttacgatgg

SEQ ID NO: 78 - DNA, 35 bp, synthetic construct
  misc_feature 1..35: note = synthetic nucleic acid
  source 1..35: mol_type = other DNA
atagcagtccagagcccgctaagatattctaagtt

SEQ ID NO: 79 - DNA, 35 bp, synthetic construct
  misc_feature 1..35: note = synthetic nucleic acid
  source 1..35: mol_type = other DNA
atagcagtccaggcgtaacgcagatgaatattcaa

SEQ ID NO: 80 - DNA, 35 bp, synthetic construct
  misc_feature 1..35: note = synthetic nucleic acid
  source 1..35: mol_type = other DNA
atagcagtccagaatttgcgtatagagcgggtcaa

SEQ ID NO: 81 - DNA, 35 bp, synthetic construct
  misc_feature 1..35: note = synthetic nucleic acid
  source 1..35: mol_type = other DNA
atagcagtccagagtaagcatctagcccggctctt

SEQ ID NO: 82 - DNA, 35 bp, synthetic construct
  misc_feature 1..35: note = synthetic nucleic acid
  source 1..35: mol_type = other DNA
atagcagtccagcgatggagattcagtctctcggg

SEQ ID NO: 83 - DNA, 35 bp, synthetic construct
  misc_feature 1..35: note = synthetic nucleic acid
  source 1..35: mol_type = other DNA
atagcagtccagcgagcactgtaataggcactatt

SEQ ID NO: 84 - DNA, 35 bp, synthetic construct
  misc_feature 1..35: note = synthetic nucleic acid
  source 1..35: mol_type = other DNA
atagcagtccagaaagagtgatgataatcatgaaa

SEQ ID NO: 85 - DNA, 35 bp, synthetic construct
  misc_feature 1..35: note = synthetic nucleic acid
  source 1..35: mol_type = other DNA
atagcagtccagggaacaaagcggtcttacggttt

SEQ ID NO: 86 - DNA, 35 bp, synthetic construct
  misc_feature 1..35: note = synthetic nucleic acid
  source 1..35: mol_type = other DNA
atagcagtccaggagaaggctgagcttggactcaa

SEQ ID NO: 87 - DNA, 35 bp, synthetic construct
  misc_feature 1..35: note = synthetic nucleic acid
  source 1..35: mol_type = other DNA
atagcagtccagaatcggatgtaggatggtctcgg

SEQ ID NO: 88 - DNA, 35 bp, synthetic construct
  misc_feature 1..35: note = synthetic nucleic acid
  source 1..35: mol_type = other DNA
atagcagtccaggtaccggacgtgccgtttcactt

SEQ ID NO: 89 - DNA, 35 bp, synthetic construct
  misc_feature 1..35: note = synthetic nucleic acid
  source 1..35: mol_type = other DNA
atagcagtccagtaccgttattgcggagcataggg

SEQ ID NO: 90 - DNA, 35 bp, synthetic construct
  misc_feature 1..35: note = synthetic nucleic acid
  source 1..35: mol_type = other DNA
atagcagtccagcttcgcggtttcctcagacacgg

SEQ ID NO: 91 - DNA, 35 bp, synthetic construct
  misc_feature 1..35: note = synthetic nucleic acid
  source 1..35: mol_type = other DNA
atagcagtccagaggcagaggcacgcccttttaaa

SEQ ID NO: 92 - DNA, 35 bp, synthetic construct
  misc_feature 1..35: note = synthetic nucleic acid
  source 1..35: mol_type = other DNA
atagcagtccagtatgattggtccactaacgtagg

SEQ ID NO: 93 - DNA, 35 bp, synthetic construct
  misc_feature 1..35: note = synthetic nucleic acid
  source 1..35: mol_type = other DNA
atagcagtccagcgcgtgatagggcatttgaaggg

SEQ ID NO: 94 - DNA, 35 bp, synthetic construct
  misc_feature 1..35: note = synthetic nucleic acid
  source 1..35: mol_type = other DNA
atagcagtccagcccgtacacatgagcgaatcagg